European Patent Specification EP 3 775 194 B1, published June 28, 2023. Title: De-immunized Factor VIII molecule and pharmaceutical compositions comprising the same. Applicant: Biotest AG. The sequence listing filed with the application follows.

SEQUENCE LISTING (54 sequences)

SEQ ID NO: 1 - protein, 2351 aa, Homo sapiens
  SIGNAL 1..19: Signal sequence
  FVIII wt full length
MQIELSTCFFLCLLRFCFSATRRYYLGAVELSWDYMQSDLGELPVDARFPPRVPKSFPFNTSVVYKKTLFVEFTDHLFNIAKPRPPWMGLLGPTIQAEVYDTVVITLKNMASHPVSLHAVGVSYWKASEGAEYDDQTSQREKEDDKVFPGGSHTYVWQVLKENGPMASDPLCLTYSYLSHVDLVKDLNSGLIGALLVCREGSLAKEKTQTLHKFILLFAVFDEGKSWHSETKNSLMQDRDAASARAWPKMHTVNGYVNRSLPGLIGCHRKSVYWHVIGMGTTPEVHSIFLEGHTFLVRNHRQASLEISPITFLTAQTLLMDLGQFLLFCHISSHQHDGMEAYVKVDSCPEEPQLRMKNNEEAEDYDDDLTDSEMDVVRFDDDNSPSFIQIRSVAKKHPKTWVHYIAAEEEDWDYAPLVLAPDDRSYKSQYLNNGPQRIGRKYKKVRFMAYTDETFKTREAIQHESGILGPLLYGEVGDTLLIIFKNQASRPYNIYPHGITDVRPLYSRRLPKGVKHLKDFPILPGEIFKYKWTVTVEDGPTKSDPRCLTRYYSSFVNMERDLASGLIGPLLICYKESVDQRGNQIMSDKRNVILFSVFDENRSWYLTENIQRFLPNPAGVQLEDPEFQASNIMHSINGYVFDSLQLSVCLHEVAYWYILSIGAQTDFLSVFFSGYTFKHKMVYEDTLTLFPFSGETVFMSMENPGLWILGCHNSDFRNRGMTALLKVSSCDKNTGDYYEDSYEDISAYLLSKNNAIEPRSFSQNSRHPSTRQKQFNATTIPENDIEKTDPWFAHRTPMPKIQNVSSSDLLMLLRQSPTPHGLSLSDLQEAKYETFSDDPSPGAIDSNNSLSEMTHFRPQLHHSGDMVFTPESGLQLRLNEKLGTTAATELKKLDFKVSSTSNNLISTIPSDNLAAGTDNTSSLGPPSMPVHYDSQLDTTLFGKKSSPLTESGGPLSLSEENNDSKLLESGLMNSQESSWGKNVSSTESGRLFKGKRAHGPALLTKDNALFKVSISLLKTNKTSNNSATNRKTHIDGPSLLIENSPSVWQNILESDTEFKKVTPLIHDRMLMDKNATALRLNHMSNKTTSSKNMEMVQQKKEGPIPPDAQNPDMSFFKMLFLPESARWIQRTHGKNSLNSGQGPSPKQLVSLGPEKSVEGQNFLSEKNKVVVGKGEFTKDVGLKEMVFPSSRNLFLTNLDNLHENNTHNQEKKIQEEIEKKETLIQENVVLPQIHTVTGTKNFMKNLFLLSTRQNVEGSYDGAYAPVLQDFRSLNDSTNRTKKHTAHFSKKGEEENLEGLGNQTKQIVEKYACTTRISPNTSQQNFVTQRSKRALKQFRLPLEETELEKRIIVDDTSTQWSKNMKHLTPSTLTQIDYNEKEKGAITQSPLSDCLTRSHSIPQANRSPLPIAKVSSFPSIRPIYLTRVLFQDNSSHLPAASYRKKDSGVQESSHFLQGAKKNNLSLAILTLEMTGDQREVGSLGTSATNSVTYKKVENTVLPKPDLPKTSGKVELLPKVHIYQKDLFPTETSNGSPGHLDLVEGSLLQGTEGAIKWNEANRPGKVPFLRVATESSAKTPSKLLDPLAWDNHYGTQIPKEEWKSQEKSPEKTAFKKKDTILSLNACESNHAIAAINEGQNKPEIEVTWAKQGRTERLCSQNPPVLKRHQREITRTTLQSDQEEIDYDDTISVEMKKEDFDIYDEDENQSPRSFQKKTRHYFIAAVERLWDYGMSSSPHVLRNRAQSGSVPQFKKVVFQEFTDGSFTQPLYRGELNEHLGLLGPYIRAEVEDNIMVTFRNQASRPYSFYSSLISYEEDQRQGAEPRKNFVKPNETKTYFWKVQHHMAPTKDEFDCKAWAYFSDVDLEKDVHSGLIGPLLVCHTNTLNPAHGRQVTVQEFALFFTIFDETKSWYFTENMERNCRAPCNIQMEDPTFKENYRFHAINGYIMDTLPGLVMAQDQRIRWYLLSMGSNENIHSIHFSGHVFTVRKKEEYKMALYNLYPGVFETVEMLPSKAGIWRVECLIGEHLHAGMSTLFLVYSNKCQTPLGMASGHIRDFQITASGQYGQWAPKLARLHYSGSINAWSTKEPFSWIKVDLLAPMIIHGIKTQGARQKFSSLYISQFIIMYSLDGKKWQTYRGNSTGTLMVFFGNVDSSGIKHNIFNPPIIARYIRLHPTHYSIRSTLRMELMGCDLNSCSMPLGMESKAISDAQITASSYFTNMFATWSPSKARLHLQGRSNAWRPQVNNPKEWLQVDFQKTMKVTGVTTQGVKSLLTSMYVKEFLISSSQDGHQWTLFFQNGKVKVFQGNQDSFTPVVNSLDPPLLTRYLRIHPQSWVHQIALRMEVLGCEAQDLY

SEQ ID NO: 2 - protein, 1533 aa, Artificial Sequence
  SIGNAL 1..19: Signal sequence
  FVIII-6rs - human FVIII B-domain deleted
  DOMAIN 20..348: A1
  DOMAIN 349..398: a1
  DOMAIN 399..730: A2
  DOMAIN 731..759: a2
  DOMAIN 760..849: truncated B-domain
  DOMAIN 850..894: a3
  DOMAIN 895..1221: A3
  DOMAIN 1222..1374: C1
  DOMAIN 1375..1533: C2
MQIELSTCFFLCLLRFCFSATRRYYLGAVELSWDYMQSDLGELPVDARFPPRVPKSFPFNTSVVYKKTLFVEFTDHLFNIAKPRPPWMGLLGPTIQAEVYDTVVITLKNMASHPVSLHAVGVSYWKASEGAEYDDQTSQREKEDDKVFPGGSHTYVWQVLKENGPMASDPLCLTYSYLSHVDLVKDLNSGLIGALLVCREGSLAKEKTQTLHKFILLFAVFDEGKSWHSETKNSLMQDRDAASARAWPKMHTVNGYVNRSLPGLIGCHRKSVYWHVIGMGTTPEVHSIFLEGHTFLVRNHRQASLEISPITFLTAQTLLMDLGQFLLFCHISSHQHDGMEAYVKVDSCPEEPQLRMKNNEEAEDYDDDLTDSEMDVVRFDDDNSPSFIQIRSVAKKHPKTWVHYIAAEEEDWDYAPLVLAPDDRSYKSQYLNNGPQRIGRKYKKVRFMAYTDETFKTREAIQHESGILGPLLYGEVGDTLLIIFKNQASRPYNIYPHGITDVRPLYSRRLPKGVKHLKDFPILPGEIFKYKWTVTVEDGPTKSDPRCLTRYYSSFVNMERDLASGLIGPLLICYKESVDQRGNQIMSDKRNVILFSVFDENRSWYLTENIQRFLPNPAGVQLEDPEFQASNIMHSINGYVFDSLQLSVCLHEVAYWYILSIGAQTDFLSVFFSGYTFKHKMVYEDTLTLFPFSGETVFMSMENPGLWILGCHNSDFRNRGMTALLKVSSCDKNTGDYYEDSYEDISAYLLSKNNAIEPRSFSQDPLAWDNHYGTQIPKEEWKSQEKSPEKTAFKKKDTILSLNACESNHAIAAINEGQNKPEIEVTWAKQGRTERLCSQNPPVLKRHQREITRTTLQSDQEEIDYDDTISVEMKKEDFDIYDEDENQSPRSFQKKTRHYFIAAVERLWDYGMSSSPHVLRNRAQSGSVPQFKKVVFQEFTDGSFTQPLYRGELNEHLGLLGPYIRAEVEDNIMVTFRNQASRPYSFYSSLISYEEDQRQGAEPRKNFVKPNETKTYFWKVQHHMAPTKDEFDCKAWAYFSDVDLEKDVHSGLIGPLLVCHTNTLNPAHGRQVTVQEFALFFTIFDETKSWYFTENMERNCRAPCNIQMEDPTFKENYRFHAINGYIMDTLPGLVMAQDQRIRWYLLSMGSNENIHSIHFSGHVFTVRKKEEYKMALYNLYPGVFETVEMLPSKAGIWRVECLIGEHLHAGMSTLFLVYSNKCQTPLGMASGHIRDFQITASGQYGQWAPKLARLHYSGSINAWSTKEPFSWIKVDLLAPMIIHGIKTQGARQKFSSLYISQFIIMYSLDGKKWQTYRGNSTGTLMVFFGNVDSSGIKHNIFNPPIIARYIRLHPTHYSIRSTLRMELMGCDLNSCSMPLGMESKAISDAQITASSYFTNMFATWSPSKARLHLQGRSNAWRPQVNNPKEWLQVDFQKTMKVTGVTTQGVKSLLTSMYVKEFLISSSQDGHQWTLFFQNGKVKVFQGNQDSFTPVVNSLDPPLLTRYLRIHPQSWVHQIALRMEVLGCEAQDLY

SEQ ID NO: 3 - protein, 1457 aa, Artificial Sequence
  Refacto - human FVIII B-domain deleted
MQIELSTCFFLCLLRFCFSATRRYYLGAVELSWDYMQSDLGELPVDARFPPRVPKSFPFNTSVVYKKTLFVEFTDHLFNIAKPRPPWMGLLGPTIQAEVYDTVVITLKNMASHPVSLHAVGVSYWKASEGAEYDDQTSQREKEDDKVFPGGSHTYVWQVLKENGPMASDPLCLTYSYLSHVDLVKDLNSGLIGALLVCREGSLAKEKTQTLHKFILLFAVFDEGKSWHSETKNSLMQDRDAASARAWPKMHTVNGYVNRSLPGLIGCHRKSVYWHVIGMGTTPEVHSIFLEGHTFLVRNHRQASLEISPITFLTAQTLLMDLGQFLLFCHISSHQHDGMEAYVKVDSCPEEPQLRMKNNEEAEDYDDDLTDSEMDVVRFDDDNSPSFIQIRSVAKKHPKTWVHYIAAEEEDWDYAPLVLAPDDRSYKSQYLNNGPQRIGRKYKKVRFMAYTDETFKTREAIQHESGILGPLLYGEVGDTLLIIFKNQASRPYNIYPHGITDVRPLYSRRLPKGVKHLKDFPILPGEIFKYKWTVTVEDGPTKSDPRCLTRYYSSFVNMERDLASGLIGPLLICYKESVDQRGNQIMSDKRNVILFSVFDENRSWYLTENIQRFLPNPAGVQLEDPEFQASNIMHSINGYVFDSLQLSVCLHEVAYWYILSIGAQTDFLSVFFSGYTFKHKMVYEDTLTLFPFSGETVFMSMENPGLWILGCHNSDFRNRGMTALLKVSSCDKNTGDYYEDSYEDISAYLLSKNNAIEPRSFSQNPPVLKRHQREITRTTLQSDQEEIDYDDTISVEMKKEDFDIYDEDENQSPRSFQKKTRHYFIAAVERLWDYGMSSSPHVLRNRAQSGSVPQFKKVVFQEFTDGSFTQPLYRGELNEHLGLLGPYIRAEVEDNIMVTFRNQASRPYSFYSSLISYEEDQRQGAEPRKNFVKPNETKTYFWKVQHHMAPTKDEFDCKAWAYFSDVDLEKDVHSGLIGPLLVCHTNTLNPAHGRQVTVQEFALFFTIFDETKSWYFTENMERNCRAPCNIQMEDPTFKENYRFHAINGYIMDTLPGLVMAQDQRIRWYLLSMGSNENIHSIHFSGHVFTVRKKEEYKMALYNLYPGVFETVEMLPSKAGIWRVECLIGEHLHAGMSTLFLVYSNKCQTPLGMASGHIRDFQITASGQYGQWAPKLARLHYSGSINAWSTKEPFSWIKVDLLAPMIIHGIKTQGARQKFSSLYISQFIIMYSLDGKKWQTYRGNSTGTLMVFFGNVDSSGIKHNIFNPPIIARYIRLHPTHYSIRSTLRMELMGCDLNSCSMPLGMESKAISDAQITASSYFTNMFATWSPSKARLHLQGRSNAWRPQVNNPKEWLQVDFQKTMKVTGVTTQGVKSLLTSMYVKEFLISSSQDGHQWTLFFQNGKVKVFQGNQDSFTPVVNSLDPPLLTRYLRIHPQSWVHQIALRMEVLGCEAQDLY

SEQ ID NO: 4 - protein, 1463 aa, Artificial Sequence
  SOURCE 1..10: Afstyla - human FVIII B-domain deleted single chain
  SIGNAL 1..19: signal sequence
MQIELSTCFFLCLLRFCFSATRRYYLGAVELSWDYMQSDLGELPVDARFPPRVPKSFPFNTSVVYKKTLFVEFTDHLFNIAKPRPPWMGLLGPTIQAEVYDTVVITLKNMASHPVSLHAVGVSYWKASEGAEYDDQTSQREKEDDKVFPGGSHTYVWQVLKENGPMASDPLCLTYSYLSHVDLVKDLNSGLIGALLVCREGSLAKEKTQTLHKFILLFAVFDEGKSWHSETKNSLMQDRDAASARAWPKMHTVNGYVNRSLPGLIGCHRKSVYWHVIGMGTTPEVHSIFLEGHTFLVRNHRQASLEISPITFLTAQTLLMDLGQFLLFCHISSHQHDGMEAYVKVDSCPEEPQLRMKNNEEAEDYDDDLTDSEMDVVRFDDDNSPSFIQIRSVAKKHPKTWVHYIAAEEEDWDYAPLVLAPDDRSYKSQYLNNGPQRIGRKYKKVRFMAYTDETFKTREAIQHESGILGPLLYGEVGDTLLIIFKNQASRPYNIYPHGITDVRPLYSRRLPKGVKHLKDFPILPGEIFKYKWTVTVEDGPTKSDPRCLTRYYSSFVNMERDLASGLIGPLLICYKESVDQRGNQIMSDKRNVILFSVFDENRSWYLTENIQRFLPNPAGVQLEDPEFQASNIMHSINGYVFDSLQLSVCLHEVAYWYILSIGAQTDFLSVFFSGYTFKHKMVYEDTLTLFPFSGETVFMSMENPGLWILGCHNSDFRNRGMTALLKVSSCDKNTGDYYEDSYEDISAYLLSKNNAIEPRSFSQNSRHPSTRQKQFNATTIPENTTLQSDQEEIDYDDTISVEMKKEDFDIYDEDENQSPRSFQKKTRHYFIAAVERLWDYGMSSSPHVLRNRAQSGSVPQFKKVVFQEFTDGSFTQPLYRGELNEHLGLLGPYIRAEVEDNIMVTFRNQASRPYSFYSSLISYEEDQRQGAEPRKNFVKPNETKTYFWKVQHHMAPTKDEFDCKAWAYFSDVDLEKDVHSGLIGPLLVCHTNTLNPAHGRQVTVQEFALFFTIFDETKSWYFTENMERNCRAPCNIQMEDPTFKENYRFHAINGYIMDTLPGLVMAQDQRIRWYLLSMGSNENIHSIHFSGHVFTVRKKEEYKMALYNLYPGVFETVEMLPSKAGIWRVECLIGEHLHAGMSTLFLVYSNKCQTPLGMASGHIRDFQITASGQYGQWAPKLARLHYSGSINAWSTKEPFSWIKVDLLAPMIIHGIKTQGARQKFSSLYISQFIIMYSLDGKKWQTYRGNSTGTLMVFFGNVDSSGIKHNIFNPPIIARYIRLHPTHYSIRSTLRMELMGCDLNSCSMPLGMESKAISDAQITASSYFTNMFATWSPSKARLHLQGRSNAWRPQVNNPKEWLQVDFQKTMKVTGVTTQGVKSLLTSMYVKEFLISSSQDGHQWTLFFQNGKVKVFQGNQDSFTPVVNSLDPPLLTRYLRIHPQSWVHQIALRMEVLGCEAQDLY

SEQ ID NO: 5 - protein, 1533 aa, Artificial Sequence
  SIGNAL 1..19
  FVIII-19M
  DOMAIN 20..348: A1
  MUTAGEN 79: N79S
  MUTAGEN 112: S112T
  MUTAGEN 160: L160S
  MUTAGEN 171: L171Q
  MUTAGEN 184: V184A
  MUTAGEN 223: N233D
  MUTAGEN 265: I265T
  MUTAGEN 299: N299D
  DOMAIN 349..398: a1
  DOMAIN 399..730: A2
  MUTAGEN 426: Y426H
  MUTAGEN 507: S507E
  MUTAGEN 555: F555H
  MUTAGEN 616: N616E
  MUTAGEN 706: L706N
  DOMAIN 731..759: a2
  MUTAGEN 748: Y748S
  DOMAIN 760..849: truncated B-domain
  DOMAIN 850..894: a3
  DOMAIN 895..1221: A3
  MUTAGEN 1019: K1837E
  MUTAGEN 1220: N2038D
  DOMAIN 1222..1374: C1
  MUTAGEN 1259: S2077G
  DOMAIN 1375..1533: C2
  MUTAGEN 1497: S2315T
  MUTAGEN 1515: V2333A
MQIELSTCFFLCLLRFCFSATRRYYLGAVELSWDYMQSDLGELPVDARFPPRVPKSFPFNTSVVYKKTLFVEFTDHLFSIAKPRPPWMGLLGPTIQAEVYDTVVITLKNMATHPVSLHAVGVSYWKASEGAEYDDQTSQREKEDDKVFPGGSHTYVWQVSKENGPMASDPQCLTYSYLSHVDLAKDLNSGLIGALLVCREGSLAKEKTQTLHKFILLFAVFDEGKSWHSETKDSLMQDRDAASARAWPKMHTVNGYVNRSLPGLTGCHRKSVYWHVIGMGTTPEVHSIFLEGHTFLVRDHRQASLEISPITFLTAQTLLMDLGQFLLFCHISSHQHDGMEAYVKVDSCPEEPQLRMKNNEEAEDYDDDLTDSEMDVVRFDDDNSPSFIQIRSVAKKHPKTWVHYIAAEEEDWDYAPLVLAPDDRSHKSQYLNNGPQRIGRKYKKVRFMAYTDETFKTREAIQHESGILGPLLYGEVGDTLLIIFKNQASRPYNIYPHGITDVRPLYERRLPKGVKHLKDFPILPGEIFKYKWTVTVEDGPTKSDPRCLTRYYSSHVNMERDLASGLIGPLLICYKESVDQRGNQIMSDKRNVILFSVFDENRSWYLTENIQRFLPEPAGVQLEDPEFQASNIMHSINGYVFDSLQLSVCLHEVAYWYILSIGAQTDFLSVFFSGYTFKHKMVYEDTLTLFPFSGETVFMSMENPGNWILGCHNSDFRNRGMTALLKVSSCDKNTGDYYEDSYEDISASLLSKNNAIEPRSFSQDPLAWDNHYGTQIPKEEWKSQEKSPEKTAFKKKDTILSLNACESNHAIAAINEGQNKPEIEVTWAKQGRTERLCSQNPPVLKRHQREITRTTLQSDQEEIDYDDTISVEMKKEDFDIYDEDENQSPRSFQKKTRHYFIAAVERLWDYGMSSSPHVLRNRAQSGSVPQFKKVVFQEFTDGSFTQPLYRGELNEHLGLLGPYIRAEVEDNIMVTFRNQASRPYSFYSSLISYEEDQRQGAEPRKNFVKPNETKTYFWEVQHHMAPTKDEFDCKAWAYFSDVDLEKDVHSGLIGPLLVCHTNTLNPAHGRQVTVQEFALFFTIFDETKSWYFTENMERNCRAPCNIQMEDPTFKENYRFHAINGYIMDTLPGLVMAQDQRIRWYLLSMGSNENIHSIHFSGHVFTVRKKEEYKMALYNLYPGVFETVEMLPSKAGIWRVECLIGEHLHAGMSTLFLVYSDKCQTPLGMASGHIRDFQITASGQYGQWAPKLARLHYSGGINAWSTKEPFSWIKVDLLAPMIIHGIKTQGARQKFSSLYISQFIIMYSLDGKKWQTYRGNSTGTLMVFFGNVDSSGIKHNIFNPPIIARYIRLHPTHYSIRSTLRMELMGCDLNSCSMPLGMESKAISDAQITASSYFTNMFATWSPSKARLHLQGRSNAWRPQVNNPKEWLQVDFQKTMKVTGVTTQGVKSLLTSMYVKEFLISSSQDGHQWTLFFQNGKVKVFQGNQDSFTPVVNTLDPPLLTRYLRIHPQSWAHQIALRMEVLGCEAQDLY

SEQ ID NO: 6 - protein, 1533 aa, Artificial Sequence
  SIGNAL 1..19
  FVIII-18M
MQIELSTCFFLCLLRFCFSATRRYYLGAVELSWDYMQSDLGELPVDARFPPRVPKSFPFNTSVVYKKTLFVEFTDHLFSIAKPRPPWMGLLGPTIQAEVYDTVVITLKNMATHPVSLHAVGVSYWKASEGAEYDDQTSQREKEDDKVFPGGSHTYVWQVSKENGPMASDPQCLTYSYLSHVDLAKDLNSGLIGALLVCREGSLAKEKTQTLHKFILLFAVFDEGKSWHSETKDSLMQDRDAASARAWPKMHTVNGYVNRSLPGLTGCHRKSVYWHVIGMGTTPEVHSIFLEGHTFLVRDHRQASLEISPITFLTAQTLLMDLGQFLLFCHISSHQHDGMEAYVKVDSCPEEPQLRMKNNEEAEDYDDDLTDSEMDVVRFDDDNSPSFIQIRSVAKKHPKTWVHYIAAEEEDWDYAPLVLAPDDRSHKSQYLNNGPQRIGRKYKKVRFMAYTDETFKTREAIQHESGILGPLLYGEVGDTLLIIFKNQASRPYNIYPHGITDVRPLYERRLPKGVKHLKDFPILPGEIFKYKWTVTVEDGPTKSDPRCLTRYYSSHVNMERDLASGLIGPLLICYKESVDQRGNQIMSDKRNVILFSVFDENRSWYLTENIQRFLPEPAGVQLEDPEFQASNIMHSINGYVFDSLQLSVCLHEVAYWYILSIGAQTDFLSVFFSGYTFKHKMVYEDTLTLFPFSGETVFMSMENPGNWILGCHNSDFRNRGMTALLKVSSCDKNTGDYYEDSYEDISASLLSKNNAIEPRSFSQDPLAWDNHYGTQIPKEEWKSQEKSPEKTAFKKKDTILSLNACESNHAIAAINEGQNKPEIEVTWAKQGRTERLCSQNPPVLKRHQREITRTTLQSDQEEIDYDDTISVEMKKEDFDIYDEDENQSPRSFQKKTRHYFIAAVERLWDYGMSSSPHVLRNRAQSGSVPQFKKVVFQEFTDGSFTQPLYRGELNEHLGLLGPYIRAEVEDNIMVTFRNQASRPYSFYSSLISYEEDQRQGAEPRKNFVKPNETKTYFWKVQHHMAPTKDEFDCKAWAYFSDVDLEKDVHSGLIGPLLVCHTNTLNPAHGRQVTVQEFALFFTIFDETKSWYFTENMERNCRAPCNIQMEDPTFKENYRFHAINGYIMDTLPGLVMAQDQRIRWYLLSMGSNENIHSIHFSGHVFTVRKKEEYKMALYNLYPGVFETVEMLPSKAGIWRVECLIGEHLHAGMSTLFLVYSDKCQTPLGMASGHIRDFQITASGQYGQWAPKLARLHYSGGINAWSTKEPFSWIKVDLLAPMIIHGIKTQGARQKFSSLYISQFIIMYSLDGKKWQTYRGNSTGTLMVFFGNVDSSGIKHNIFNPPIIARYIRLHPTHYSIRSTLRMELMGCDLNSCSMPLGMESKAISDAQITASSYFTNMFATWSPSKARLHLQGRSNAWRPQVNNPKEWLQVDFQKTMKVTGVTTQGVKSLLTSMYVKEFLISSSQDGHQWTLFFQNGKVKVFQGNQDSFTPVVNTLDPPLLTRYLRIHPQSWAHQIALRMEVLGCEAQDLY

SEQ ID NO: 7 - protein, 1533 aa, Artificial Sequence
  SIGNAL 1..19
  FVIII-15M
MQIELSTCFFLCLLRFCFSATRRYYLGAVELSWDYMQSDLGELPVDARFPPRVPKSFPFNTSVVYKKTLFVEFTDHLFSIAKPRPPWMGLLGPTIQAEVYDTVVITLKNMATHPVSLHAVGVSYWKASEGAEYDDQTSQREKEDDKVFPGGSHTYVWQVSKENGPMASDPQCLTYSYLSHVDLAKDLNSGLIGALLVCREGSLAKEKTQTLHKFILLFAVFDEGKSWHSETKDSLMQDRDAASARAWPKMHTVNGYVNRSLPGLTGCHRKSVYWHVIGMGTTPEVHSIFLEGHTFLVRDHRQASLEISPITFLTAQTLLMDLGQFLLFCHISSHQHDGMEAYVKVDSCPEEPQLRMKNNEEAEDYDDDLTDSEMDVVRFDDDNSPSFIQIRSVAKKHPKTWVHYIAAEEEDWDYAPLVLAPDDRSHKSQYLNNGPQRIGRKYKKVRFMAYTDETFKTREAIQHESGILGPLLYGEVGDTLLIIFKNQASRPYNIYPHGITDVRPLYERRLPKGVKHLKDFPILPGEIFKYKWTVTVEDGPTKSDPRCLTRYYSSHVNMERDLASGLIGPLLICYKESVDQRGNQIMSDKRNVILFSVFDENRSWYLTENIQRFLPEPAGVQLEDPEFQASNIMHSINGYVFDSLQLSVCLHEVAYWYILSIGAQTDFLSVFFSGYTFKHKMVYEDTLTLFPFSGETVFMSMENPGNWILGCHNSDFRNRGMTALLKVSSCDKNTGDYYEDSYEDISASLLSKNNAIEPRSFSQDPLAWDNHYGTQIPKEEWKSQEKSPEKTAFKKKDTILSLNACESNHAIAAINEGQNKPEIEVTWAKQGRTERLCSQNPPVLKRHQREITRTTLQSDQEEIDYDDTISVEMKKEDFDIYDEDENQSPRSFQKKTRHYFIAAVERLWDYGMSSSPHVLRNRAQSGSVPQFKKVVFQEFTDGSFTQPLYRGELNEHLGLLGPYIRAEVEDNIMVTFRNQASRPYSFYSSLISYEEDQRQGAEPRKNFVKPNETKTYFWEVQHHMAPTKDEFDCKAWAYFSDVDLEKDVHSGLIGPLLVCHTNTLNPAHGRQVTVQEFALFFTIFDETKSWYFTENMERNCRAPCNIQMEDPTFKENYRFHAINGYIMDTLPGLVMAQDQRIRWYLLSMGSNENIHSIHFSGHVFTVRKKEEYKMALYNLYPGVFETVEMLPSKAGIWRVECLIGEHLHAGMSTLFLVYSNKCQTPLGMASGHIRDFQITASGQYGQWAPKLARLHYSGSINAWSTKEPFSWIKVDLLAPMIIHGIKTQGARQKFSSLYISQFIIMYSLDGKKWQTYRGNSTGTLMVFFGNVDSSGIKHNIFNPPIIARYIRLHPTHYSIRSTLRMELMGCDLNSCSMPLGMESKAISDAQITASSYFTNMFATWSPSKARLHLQGRSNAWRPQVNNPKEWLQVDFQKTMKVTGVTTQGVKSLLTSMYVKEFLISSSQDGHQWTLFFQNGKVKVFQGNQDSFTPVVNSLDPPLLTRYLRIHPQSWVHQIALRMEVLGCEAQDLY

SEQ ID NO: 8 - protein, 1533 aa, Artificial Sequence
  SIGNAL 1..19
  FVIII-A1-7M
MQIELSTCFFLCLLRFCFSATRRYYLGAVELSWDYMQSDLGELPVDARFPPRVPKSFPFNTSVVYKKTLFVEFTDHLFSIAKPRPPWMGLLGPTIQAEVYDTVVITLKNMATHPVSLHAVGVSYWKASEGAEYDDQTSQREKEDDKVFPGGSHTYVWQVSKENGPMASDPQCLTYSYLSHVDLAKDLNSGLIGALLVCREGSLAKEKTQTLHKFILLFAVFDEGKSWHSETKDSLMQDRDAASARAWPKMHTVNGYVNRSLPGLTGCHRKSVYWHVIGMGTTPEVHSIFLEGHTFLVRNHRQASLEISPITFLTAQTLLMDLGQFLLFCHISSHQHDGMEAYVKVDSCPEEPQLRMKNNEEAEDYDDDLTDSEMDVVRFDDDNSPSFIQIRSVAKKHPKTWVHYIAAEEEDWDYAPLVLAPDDRSYKSQYLNNGPQRIGRKYKKVRFMAYTDETFKTREAIQHESGILGPLLYGEVGDTLLIIFKNQASRPYNIYPHGITDVRPLYSRRLPKGVKHLKDFPILPGEIFKYKWTVTVEDGPTKSDPRCLTRYYSSFVNMERDLASGLIGPLLICYKESVDQRGNQIMSDKRNVILFSVFDENRSWYLTENIQRFLPNPAGVQLEDPEFQASNIMHSINGYVFDSLQLSVCLHEVAYWYILSIGAQTDFLSVFFSGYTFKHKMVYEDTLTLFPFSGETVFMSMENPGLWILGCHNSDFRNRGMTALLKVSSCDKNTGDYYEDSYEDISAYLLSKNNAIEPRSFSQDPLAWDNHYGTQIPKEEWKSQEKSPEKTAFKKKDTILSLNACESNHAIAAINEGQNKPEIEVTWAKQGRTERLCSQNPPVLKRHQREITRTTLQSDQEEIDYDDTISVEMKKEDFDIYDEDENQSPRSFQKKTRHYFIAAVERLWDYGMSSSPHVLRNRAQSGSVPQFKKVVFQEFTDGSFTQPLYRGELNEHLGLLGPYIRAEVEDNIMVTFRNQASRPYSFYSSLISYEEDQRQGAEPRKNFVKPNETKTYFWKVQHHMAPTKDEFDCKAWAYFSDVDLEKDVHSGLIGPLLVCHTNTLNPAHGRQVTVQEFALFFTIFDETKSWYFTENMERNCRAPCNIQMEDPTFKENYRFHAINGYIMDTLPGLVMAQDQRIRWYLLSMGSNENIHSIHFSGHVFTVRKKEEYKMALYNLYPGVFETVEMLPSKAGIWRVECLIGEHLHAGMSTLFLVYSNKCQTPLGMASGHIRDFQITASGQYGQWAPKLARLHYSGSINAWSTKEPFSWIKVDLLAPMIIHGIKTQGARQKFSSLYISQFIIMYSLDGKKWQTYRGNSTGTLMVFFGNVDSSGIKHNIFNPPIIARYIRLHPTHYSIRSTLRMELMGCDLNSCSMPLGMESKAISDAQITASSYFTNMFATWSPSKARLHLQGRSNAWRPQVNNPKEWLQVDFQKTMKVTGVTTQGVKSLLTSMYVKEFLISSSQDGHQWTLFFQNGKVKVFQGNQDSFTPVVNSLDPPLLTRYLRIHPQSWVHQIALRMEVLGCEAQDLY

SEQ ID NO: 9 - protein, 1533 aa, Artificial Sequence
  SIGNAL 1..19
  FVIII-A2-4M
MQIELSTCFFLCLLRFCFSATRRYYLGAVELSWDYMQSDLGELPVDARFPPRVPKSFPFNTSVVYKKTLFVEFTDHLFNIAKPRPPWMGLLGPTIQAEVYDTVVITLKNMASHPVSLHAVGVSYWKASEGAEYDDQTSQREKEDDKVFPGGSHTYVWQVLKENGPMASDPLCLTYSYLSHVDLVKDLNSGLIGALLVCREGSLAKEKTQTLHKFILLFAVFDEGKSWHSETKNSLMQDRDAASARAWPKMHTVNGYVNRSLPGLIGCHRKSVYWHVIGMGTTPEVHSIFLEGHTFLVRNHRQASLEISPITFLTAQTLLMDLGQFLLFCHISSHQHDGMEAYVKVDSCPEEPQLRMKNNEEAEDYDDDLTDSEMDVVRFDDDNSPSFIQIRSVAKKHPKTWVHYIAAEEEDWDYAPLVLAPDDRSYKSQYLNNGPQRIGRKYKKVRFMAYTDETFKTREAIQHESGILGPLLYGEVGDTLLIIFKNQASRPYNIYPHGITDVRPLYSRRLPKGVKHLKDFPILPGEIFKYKWTVTVEDGPTKSDPRCLTRYYSSHVNMERDLASGLIGPLLICYKESVDQRGNQIMSDKRNVILFSVFDENRSWYLTENIQRFLPEPAGVQLEDPEFQASNIMHSINGYVFDSLQLSVCLHEVAYWYILSIGAQTDFLSVFFSGYTFKHKMVYEDTLTLFPFSGETVFMSMENPGNWILGCHNSDFRNRGMTALLKVSSCDKNTGDYYEDSYEDISASLLSKNNAIEPRSFSQDPLAWDNHYGTQIPKEEWKSQEKSPEKTAFKKKDTILSLNACESNHAIAAINEGQNKPEIEVTWAKQGRTERLCSQNPPVLKRHQREITRTTLQSDQEEIDYDDTISVEMKKEDFDIYDEDENQSPRSFQKKTRHYFIAAVERLWDYGMSSSPHVLRNRAQSGSVPQFKKVVFQEFTDGSFTQPLYRGELNEHLGLLGPYIRAEVEDNIMVTFRNQASRPYSFYSSLISYEEDQRQGAEPRKNFVKPNETKTYFWKVQHHMAPTKDEFDCKAWAYFSDVDLEKDVHSGLIGPLLVCHTNTLNPAHGRQVTVQEFALFFTIFDETKSWYFTENMERNCRAPCNIQMEDPTFKENYRFHAINGYIMDTLPGLVMAQDQRIRWYLLSMGSNENIHSIHFSGHVFTVRKKEEYKMALYNLYPGVFETVEMLPSKAGIWRVECLIGEHLHAGMSTLFLVYSNKCQTPLGMASGHIRDFQITASGQYGQWAPKLARLHYSGSINAWSTKEPFSWIKVDLLAPMIIHGIKTQGARQKFSSLYISQFIIMYSLDGKKWQTYRGNSTGTLMVFFGNVDSSGIKHNIFNPPIIARYIRLHPTHYSIRSTLRMELMGCDLNSCSMPLGMESKAISDAQITASSYFTNMFATWSPSKARLHLQGRSNAWRPQVNNPKEWLQVDFQKTMKVTGVTTQGVKSLLTSMYVKEFLISSSQDGHQWTLFFQNGKVKVFQGNQDSFTPVVNSLDPPLLTRYLRIHPQSWVHQIALRMEVLGCEAQDLY

SEQ ID NO: 10 - protein, 1533 aa, Artificial Sequence
  SIGNAL 1..19
  FVIII-BA3-1M
MQIELSTCFFLCLLRFCFSATRRYYLGAVELSWDYMQSDLGELPVDARFPPRVPKSFPFNTSVVYKKTLFVEFTDHLFNIAKPRPPWMGLLGPTIQAEVYDTVVITLKNMASHPVSLHAVGVSYWKASEGAEYDDQTSQREKEDDKVFPGGSHTYVWQVLKENGPMASDPLCLTYSYLSHVDLVKDLNSGLIGALLVCREGSLAKEKTQTLHKFILLFAVFDEGKSWHSETKNSLMQDRDAASARAWPKMHTVNGYVNRSLPGLIGCHRKSVYWHVIGMGTTPEVHSIFLEGHTFLVRNHRQASLEISPITFLTAQTLLMDLGQFLLFCHISSHQHDGMEAYVKVDSCPEEPQLRMKNNEEAEDYDDDLTDSEMDVVRFDDDNSPSFIQIRSVAKKHPKTWVHYIAAEEEDWDYAPLVLAPDDRSYKSQYLNNGPQRIGRKYKKVRFMAYTDETFKTREAIQHESGILGPLLYGEVGDTLLIIFKNQASRPYNIYPHGITDVRPLYSRRLPKGVKHLKDFPILPGEIFKYKWTVTVEDGPTKSDPRCLTRYYSSFVNMERDLASGLIGPLLICYKESVDQRGNQIMSDKRNVILFSVFDENRSWYLTENIQRFLPNPAGVQLEDPEFQASNIMHSINGYVFDSLQLSVCLHEVAYWYILSIGAQTDFLSVFFSGYTFKHKMVYEDTLTLFPFSGETVFMSMENPGLWILGCHNSDFRNRGMTALLKVSSCDKNTGDYYEDSYEDISAYLLSKNNAIEPRSFSQDPLAWDNHYGTQIPKEEWKSQEKSPEKTAFKKKDTILSLNACESNHAIAAINEGQNKPEIEVTWAKQGRTERLCSQNPPVLKRHQREITRTTLQSDQEEIDYDDTISVEMKKEDFDIYDEDENQSPRSFQKKTRHYFIAAVERLWDYGMSSSPHVLRNRAQSGSVPQFKKVVFQEFTDGSFTQPLYRGELNEHLGLLGPYIRAEVEDNIMVTFRNQASRPYSFYSSLISYEEDQRQGAEPRKNFVKPNETKTYFWEVQHHMAPTKDEFDCKAWAYFSDVDLEKDVHSGLIGPLLVCHTNTLNPAHGRQVTVQEFALFFTIFDETKSWYFTENMERNCRAPCNIQMEDPTFKENYRFHAINGYIMDTLPGLVMAQDQRIRWYLLSMGSNENIHSIHFSGHVFTVRKKEEYKMALYNLYPGVFETVEMLPSKAGIWRVECLIGEHLHAGMSTLFLVYSNKCQTPLGMASGHIRDFQITASGQYGQWAPKLARLHYSGSINAWSTKEPFSWIKVDLLAPMIIHGIKTQGARQKFSSLYISQFIIMYSLDGKKWQTYRGNSTGTLMVFFGNVDSSGIKHNIFNPPIIARYIRLHPTHYSIRSTLRMELMGCDLNSCSMPLGMESKAISDAQITASSYFTNMFATWSPSKARLHLQGRSNAWRPQVNNPKEWLQVDFQKTMKVTGVTTQGVKSLLTSMYVKEFLISSSQDGHQWTLFFQNGKVKVFQGNQDSFTPVVNSLDPPLLTRYLRIHPQSWVHQIALRMEVLGCEAQDLY

SEQ ID NO: 11 - protein, 1533 aa, Artificial Sequence
  SIGNAL 1..19
  FVIII-A3C2-4M
MQIELSTCFFLCLLRFCFSATRRYYLGAVELSWDYMQSDLGELPVDARFPPRVPKSFPFNTSVVYKKTLFVEFTDHLFNIAKPRPPWMGLLGPTIQAEVYDTVVITLKNMASHPVSLHAVGVSYWKASEGAEYDDQTSQREKEDDKVFPGGSHTYVWQVLKENGPMASDPLCLTYSYLSHVDLVKDLNSGLIGALLVCREGSLAKEKTQTLHKFILLFAVFDEGKSWHSETKNSLMQDRDAASARAWPKMHTVNGYVNRSLPGLIGCHRKSVYWHVIGMGTTPEVHSIFLEGHTFLVRNHRQASLEISPITFLTAQTLLMDLGQFLLFCHISSHQHDGMEAYVKVDSCPEEPQLRMKNNEEAEDYDDDLTDSEMDVVRFDDDNSPSFIQIRSVAKKHPKTWVHYIAAEEEDWDYAPLVLAPDDRSYKSQYLNNGPQRIGRKYKKVRFMAYTDETFKTREAIQHESGILGPLLYGEVGDTLLIIFKNQASRPYNIYPHGITDVRPLYSRRLPKGVKHLKDFPILPGEIFKYKWTVTVEDGPTKSDPRCLTRYYSSFVNMERDLASGLIGPLLICYKESVDQRGNQIMSDKRNVILFSVFDENRSWYLTENIQRFLPNPAGVQLEDPEFQASNIMHSINGYVFDSLQLSVCLHEVAYWYILSIGAQTDFLSVFFSGYTFKHKMVYEDTLTLFPFSGETVFMSMENPGLWILGCHNSDFRNRGMTALLKVSSCDKNTGDYYEDSYEDISAYLLSKNNAIEPRSFSQDPLAWDNHYGTQIPKEEWKSQEKSPEKTAFKKKDTILSLNACESNHAIAAINEGQNKPEIEVTWAKQGRTERLCSQNPPVLKRHQREITRTTLQSDQEEIDYDDTISVEMKKEDFDIYDEDENQSPRSFQKKTRHYFIAAVERLWDYGMSSSPHVLRNRAQSGSVPQFKKVVFQEFTDGSFTQPLYRGELNEHLGLLGPYIRAEVEDNIMVTFRNQASRPYSFYSSLISYEEDQRQGAEPRKNFVKPNETKTYFWKVQHHMAPTKDEFDCKAWAYFSDVDLEKDVHSGLIGPLLVCHTNTLNPAHGRQVTVQEFALFFTIFDETKSWYFTENMERNCRAPCNIQMEDPTFKENYRFHAINGYIMDTLPGLVMAQDQRIRWYLLSMGSNENIHSIHFSGHVFTVRKKEEYKMALYNLYPGVFETVEMLPSKAGIWRVECLIGEHLHAGMSTLFLVYSDKCQTPLGMASGHIRDFQITASGQYGQWAPKLARLHYSGGINAWSTKEPFSWIKVDLLAPMIIHGIKTQGARQKFSSLYISQFIIMYSLDGKKWQTYRGNSTGTLMVFFGNVDSSGIKHNIFNPPIIARYIRLHPTHYSIRSTLRMELMGCDLNSCSMPLGMESKAISDAQITASSYFTNMFATWSPSKARLHLQGRSNAWRPQVNNPKEWLQVDFQKTMKVTGVTTQGVKSLLTSMYVKEFLISSSQDGHQWTLFFQNGKVKVFQGNQDSFTPVVNTLDPPLLTRYLRIHPQSWAHQIALRMEVLGCEAQDLY

SEQ ID NO: 12 - protein, 1533 aa, Artificial Sequence
  SIGNAL 1..19
  FVIII-GOF1
MQIELSTCFFLCLLRFCFSATRRYYLGAVELSWDYMQSDLGELPVDARFPPRVPKSFPFNTSVVYKKTLFVEFTDHLFNIAKPRPPWMGLLGPTIQAEVYDTVVITLKNMASHPVSLHAVGVSYWKASEGAEYDDQTSQREKEDDKVFPGGSHTYVWQVLKENGPMASDPQCLTYSYLSHVDLVKDLNSGLIGALLVCREGSLAKEKTQTLHKFILLFAVFDEGKSWHSETKNSLMQDRDAASARAWPKMHTVNGYVNRSLPGLIGCHRKSVYWHVIGMGTTPEVHSIFLEGHTFLVRNHRQASLEISPITFLTAQTLLMDLGQFLLFCHISSHQHDGMEAYVKVDSCPEEPQLRMKNNEEAEDYDDDLTDSEMDVVRFDDDNSPSFIQIRSVAKKHPKTWVHYIAAEEEDWDYAPLVLAPDDRSYKSQYLNNGPQRIGRKYKKVRFMAYTDETFKTREAIQHESGILGPLLYGEVGDTLLIIFKNQASRPYNIYPHGITDVRPLYERRLPKGVKHLKDFPILPGEIFKYKWTVTVEDGPTKSDPRCLTRYYSSFVNMERDLASGLIGPLLICYKESVDQRGNQIMSDKRNVILFSVFDENRSWYLTENIQRFLPNPAGVQLEDPEFQASNIMHSINGYVFDSLQLSVCLHEVAYWYILSIGAQTDFLSVFFSGYTFKHKMVYEDTLTLFPFSGETVFMSMENPGLWILGCHNSDFRNRGMTALLKVSSCDKNTGDYYEDSYEDISASLLSKNNAIEPRSFSQDPLAWDNHYGTQIPKEEWKSQEKSPEKTAFKKKDTILSLNACESNHAIAAINEGQNKPEIEVTWAKQGRTERLCSQNPPVLKRHQREITRTTLQSDQEEIDYDDTISVEMKKEDFDIYDEDENQSPRSFQKKTRHYFIAAVERLWDYGMSSSPHVLRNRAQSGSVPQFKKVVFQEFTDGSFTQPLYRGELNEHLGLLGPYIRAEVEDNIMVTFRNQASRPYSFYSSLISYEEDQRQGAEPRKNFVKPNETKTYFWKVQHHMAPTKDEFDCKAWAYFSDVDLEKDVHSGLIGPLLVCHTNTLNPAHGRQVTVQEFALFFTIFDETKSWYFTENMERNCRAPCNIQMEDPTFKENYRFHAINGYIMDTLPGLVMAQDQRIRWYLLSMGSNENIHSIHFSGHVFTVRKKEEYKMALYNLYPGVFETVEMLPSKAGIWRVECLIGEHLHAGMSTLFLVYSNKCQTPLGMASGHIRDFQITASGQYGQWAPKLARLHYSGSINAWSTKEPFSWIKVDLLAPMIIHGIKTQGARQKFSSLYISQFIIMYSLDGKKWQTYRGNSTGTLMVFFGNVDSSGIKHNIFNPPIIARYIRLHPTHYSIRSTLRMELMGCDLNSCSMPLGMESKAISDAQITASSYFTNMFATWSPSKARLHLQGRSNAWRPQVNNPKEWLQVDFQKTMKVTGVTTQGVKSLLTSMYVKEFLISSSQDGHQWTLFFQNGKVKVFQGNQDSFTPVVNSLDPPLLTRYLRIHPQSWAHQIALRMEVLGCEAQDLY

SEQ ID NO: 13 - protein, 1533 aa, Artificial Sequence
  SIGNAL 1..19
  FVIII-GOF2
MQIELSTCFFLCLLRFCFSATRRYYLGAVELSWDYMQSDLGELPVDARFPPRVPKSFPFNTSVVYKKTLFVEFTDHLFNIAKPRPPWMGLLGPTIQAEVYDTVVITLKNMASHPVSLHAVGVSYWKASEGAEYDDQTSQREKEDDKVFPGGSHTYVWQVLKENGPMASDPQCLTYSYLSHVDLVKDLNSGLIGALLVCREGSLAKEKTQTLHKFILLFAVFDEGKSWHSETKNSLMQDRDAASARAWPKMHTVNGYVNRSLPGLIGCHRKSVYWHVIGMGTTPEVHSIFLEGHTFLVRDHRQASLEISPITFLTAQTLLMDLGQFLLFCHISSHQHDGMEAYVKVDSCPEEPQLRMKNNEEAEDYDDDLTDSEMDVVRFDDDNSPSFIQIRSVAKKHPKTWVHYIAAEEEDWDYAPLVLAPDDRSYKSQYLNNGPQRIGRKYKKVRFMAYTDETFKTREAIQHESGILGPLLYGEVGDTLLIIFKNQASRPYNIYPHGITDVRPLYSRRLPKGVKHLKDFPILPGEIFKYKWTVTVEDGPTKSDPRCLTRYYSSFVNMERDLASGLIGPLLICYKESVDQRGNQIMSDKRNVILFSVFDENRSWYLTENIQRFLPEPAGVQLEDPEFQASNIMHSINGYVFDSLQLSVCLHEVAYWYILSIGAQTDFLSVFFSGYTFKHKMVYEDTLTLFPFSGETVFMSMENPGLWILGCHNSDFRNRGMTALLKVSSCDKNTGDYYEDSYEDISAYLLSKNNAIEPRSFSQDPLAWDNHYGTQIPKEEWKSQEKSPEKTAFKKKDTILSLNACESNHAIAAINEGQNKPEIEVTWAKQGRTERLCSQNPPVLKRHQREITRTTLQSDQEEIDYDDTISVEMKKEDFDIYDEDENQSPRSFQKKTRHYFIAAVERLWDYGMSSSPHVLRNRAQSGSVPQFKKVVFQEFTDGSFTQPLYRGELNEHLGLLGPYIRAEVEDNIMVTFRNQASRPYSFYSSLISYEEDQRQGAEPRKNFVKPNETKTYFWKVQHHMAPTKDEFDCKAWAYFSDVDLEKDVHSGLIGPLLVCHTNTLNPAHGRQVTVQEFALFFTIFDETKSWYFTENMERNCRAPCNIQMEDPTFKENYRFHAINGYIMDTLPGLVMAQDQRIRWYLLSMGSNENIHSIHFSGHVFTVRKKEEYKMALYNLYPGVFETVEMLPSKAGIWRVECLIGEHLHAGMSTLFLVYSNKCQTPLGMASGHIRDFQITASGQYGQWAPKLARLHYSGSINAWSTKEPFSWIKVDLLAPMIIHGIKTQGARQKFSSLYISQFIIMYSLDGKKWQTYRGNSTGTLMVFFGNVDSSGIKHNIFNPPIIARYIRLHPTHYSIRSTLRMELMGCDLNSCSMPLGMESKAISDAQITASSYFTNMFATWSPSKARLHLQGRSNAWRPQVNNPKEWLQVDFQKTMKVTGVTTQGVKSLLTSMYVKEFLISSSQDGHQWTLFFQNGKVKVFQGNQDSFTPVVNSLDPPLLTRYLRIHPQSWAHQIALRMEVLGCEAQDLY

SEQ ID NO: 14 - protein, 1533 aa, Artificial Sequence
  SIGNAL 1..19
  FVIII-LS1
MQIELSTCFFLCLLRFCFSATRRYYLGAVELSWDYMQSDLGELPVDARFPPRVPKSFPFNTSVVYKKTLFVEFTDHLFNIAKPRPPWMGLLGPTIQAEVYDTVVITLKNMATHPVSLHAVGVSYWKASEGAEYDDQTSQREKEDDKVFPGGSHTYVWQVLKENGPMASDPLCLTYSYLSHVDLVKDLNSGLIGALLVCREGSLAKEKTQTLHKFILLFAVFDEGKSWHSETKNSLMQDRDAASARAWPKMHTVNGYVNRSLPGLIGCHRKSVYWHVIGMGTTPEVHSIFLEGHTFLVRNHRQASLEISPITFLTAQTLLMDLGQFLLFCHISSHQHDGMEAYVKVDSCPEEPQLRMKNNEEAEDYDDDLTDSEMDVVRFDDDNSPSFIQIRSVAKKHPKTWVHYIAAEEEDWDYAPLVLAPDDRSYKSQYLNNGPQRIGRKYKKVRFMAYTDETFKTREAIQHESGILGPLLYGEVGDTLLIIFKNQASRPYNIYPHGITDVRPLYERRLPKGVKHLKDFPILPGEIFKYKWTVTVEDGPTKSDPRCLTRYYSSFVNMERDLASGLIGPLLICYKESVDQRGNQIMSDKRNVILFSVFDENRSWYLTENIQRFLPNPAGVQLEDPEFQASNIMHSINGYVFDSLQLSVCLHEVAYWYILSIGAQTDFLSVFFSGYTFKHKMVYEDTLTLFPFSGETVFMSMENPGLWILGCHNSDFRNRGMTALLKVSSCDKNTGDYYEDSYEDISASLLSKNNAIEPRSFSQDPLAWDNHYGTQIPKEEWKSQEKSPEKTAFKKKDTILSLNACESNHAIAAINEGQNKPEIEVTWAKQGRTERLCSQNPPVLKRHQREITRTTLQSDQEEIDYDDTISVEMKKEDFDIYDEDENQSPRSFQKKTRHYFIAAVERLWDYGMSSSPHVLRNRAQSGSVPQFKKVVFQEFTDGSFTQPLYRGELNEHLGLLGPYIRAEVEDNIMVTFRNQASRPYSFYSSLISYEEDQRQGAEPRKNFVKPNETKTYFWEVQHHMAPTKDEFDCKAWAYFSDVDLEKDVHSGLIGPLLVCHTNTLNPAHGRQVTVQEFALFFTIFDETKSWYFTENMERNCRAPCNIQMEDPTFKENYRFHAINGYIMDTLPGLVMAQDQRIRWYLLSMGSNENIHSIHFSGHVFTVRKKEEYKMALYNLYPGVFETVEMLPSKAGIWRVECLIGEHLHAGMSTLFLVYSDKCQTPLGMASGHIRDFQITASGQYGQWAPKLARLHYSGSINAWSTKEPFSWIKVDLLAPMIIHGIKTQGARQKFSSLYISQFIIMYSLDGKKWQTYRGNSTGTLMVFFGNVDSSGIKHNIFNPPIIARYIRLHPTHYSIRSTLRMELMGCDLNSCSMPLGMESKAISDAQITASSYFTNMFATWSPSKARLHLQGRSNAWRPQVNNPKEWLQVDFQKTMKVTGVTTQGVKSLLTSMYVKEFLISSSQDGHQWTLFFQNGKVKVFQGNQDSFTPVVNSLDPPLLTRYLRIHPQSWVHQIALRMEVLGCEAQDLY

SEQ ID NO: 15 - protein, 1533 aa, Artificial Sequence
  SIGNAL 1..19
  FVIII-LS2
  MUTAGEN 112: S112T
  MUTAGEN 426: Y426H
  MUTAGEN 754: N754D
  MUTAGEN 1019: K1837E
  MUTAGEN 1220: N2038D
MQIELSTCFFLCLLRFCFSATRRYYLGAVELSWDYMQSDLGELPVDARFPPRVPKSFPFNTSVVYKKTLFVEFTDHLFNIAKPRPPWMGLLGPTIQAEVYDTVVITLKNMATHPVSLHAVGVSYWKASEGAEYDDQTSQREKEDDKVFPGGSHTYVWQVLKENGPMASDPLCLTYSYLSHVDLVKDLNSGLIGALLVCREGSLAKEKTQTLHKFILLFAVFDEGKSWHSETKNSLMQDRDAASARAWPKMHTVNGYVNRSLPGLIGCHRKSVYWHVIGMGTTPEVHSIFLEGHTFLVRNHRQASLEISPITFLTAQTLLMDLGQFLLFCHISSHQHDGMEAYVKVDSCPEEPQLRMKNNEEAEDYDDDLTDSEMDVVRFDDDNSPSFIQIRSVAKKHPKTWVHYIAAEEEDWDYAPLVLAPDDRSHKSQYLNNGPQRIGRKYKKVRFMAYTDETFKTREAIQHESGILGPLLYGEVGDTLLIIFKNQASRPYNIYPHGITDVRPLYSRRLPKGVKHLKDFPILPGEIFKYKWTVTVEDGPTKSDPRCLTRYYSSFVNMERDLASGLIGPLLICYKESVDQRGNQIMSDKRNVILFSVFDENRSWYLTENIQRFLPNPAGVQLEDPEFQASNIMHSINGYVFDSLQLSVCLHEVAYWYILSIGAQTDFLSVFFSGYTFKHKMVYEDTLTLFPFSGETVFMSMENPGLWILGCHNSDFRNRGMTALLKVSSCDKNTGDYYEDSYEDISAYLLSKNDAIEPRSFSQDPLAWDNHYGTQIPKEEWKSQEKSPEKTAFKKKDTILSLNACESNHAIAAINEGQNKPEIEVTWAKQGRTERLCSQNPPVLKRHQREITRTTLQSDQEEIDYDDTISVEMKKEDFDIYDEDENQSPRSFQKKTRHYFIAAVERLWDYGMSSSPHVLRNRAQSGSVPQFKKVVFQEFTDGSFTQPLYRGELNEHLGLLGPYIRAEVEDNIMVTFRNQASRPYSFYSSLISYEEDQRQGAEPRKNFVKPNETKTYFWEVQHHMAPTKDEFDCKAWAYFSDVDLEKDVHSGLIGPLLVCHTNTLNPAHGRQVTVQEFALFFTIFDETKSWYFTENMERNCRAPCNIQMEDPTFKENYRFHAINGYIMDTLPGLVMAQDQRIRWYLLSMGSNENIHSIHFSGHVFTVRKKEEYKMALYNLYPGVFETVEMLPSKAGIWRVECLIGEHLHAGMSTLFLVYSDKCQTPLGMASGHIRDFQITASGQYGQWAPKLARLHYSGSINAWSTKEPFSWIKVDLLAPMIIHGIKTQGARQKFSSLYISQFIIMYSLDGKKWQTYRGNSTGTLMVFFGNVDSSGIKHNIFNPPIIARYIRLHPTHYSIRSTLRMELMGCDLNSCSMPLGMESKAISDAQITASSYFTNMFATWSPSKARLHLQGRSNAWRPQVNNPKEWLQVDFQKTMKVTGVTTQGVKSLLTSMYVKEFLISSSQDGHQWTLFFQNGKVKVFQGNQDSFTPVVNSLDPPLLTRYLRIHPQSWVHQIALRMEVLGCEAQDLY

SEQ ID NO: 16 - protein, 15 aa, Homo sapiens
  Immunogenic cluster identified in FVIII
DHLFNIAKPRPPWMG

SEQ ID NO: 17 - protein, 18 aa, Homo sapiens
  Immunogenic cluster identified in FVIII
YDTVVITLKNMASHPVSL

SEQ ID NO: 18 - protein, 16 aa, Homo sapiens
  Immunogenic cluster identified in FVIII
VWQVLKENGPMASDPL

SEQ ID NO: 19 - protein, 18 aa, Homo sapiens
  Immunogenic cluster identified in FVIII
SDPLCLTYSYLSHVDLVK

SEQ ID NO: 20 - protein, 16 aa, Homo sapiens
  Immunogenic cluster identified in FVIII
HVDLVKDLNSGLIGAL

SEQ ID NO: 21 - protein, 18 aa, Homo sapiens
  Immunogenic cluster identified in FVIII
TQTLHKFILLFAVFDEGK

SEQ ID NO: 22 - protein, 15 aa, Homo sapiens
  Immunogenic cluster identified in FVIII
GKSWHSETKNSLMQD

SEQ ID NO: 23 - protein, 17 aa, Homo sapiens
  Immunogenic cluster identified in FVIII
MHTVNGYVNRSLPGLIG

SEQ ID NO: 24 - protein, 17 aa, Homo sapiens
  Immunogenic cluster identified in FVIII
GHTFLVRNHRQASLEIS

SEQ ID NO: 25 - protein, 17 aa, Homo sapiens
  Immunogenic cluster identified in FVIII
ISPITFLTAQTLLMDLG

SEQ ID NO: 26 - protein, 19 aa, Homo sapiens
  Immunogenic cluster identified in FVIII
DRSYKSQYLNNGPQRIGRK

SEQ ID NO: 27 - protein, 19 aa, Homo sapiens
  Immunogenic cluster identified in FVIII
GDTLLIIFKNQASRPYNIY

SEQ ID NO: 28 - protein, 19 aa, Homo sapiens
  Immunogenic cluster identified in FVIII
ITDVRPLYSRRLPKGVKHL

SEQ ID NO: 29 - protein, 22 aa, Homo sapiens
  Immunogenic cluster identified in FVIII
PRCLTRYYSSFVNMERDLASGL

SEQ ID NO: 30 - protein, 18 aa, Homo sapiens
  Immunogenic cluster identified in FVIII
TENIQRFLPNPAGVQLED

SEQ ID NO: 31 - protein, 19 aa, Homo sapiens
  Immunogenic cluster identified in FVIII
PEFQASNIMHSINGYVFDS

SEQ ID NO: 32 - protein, 17 aa, Homo sapiens
  Immunogenic cluster identified in FVIII
EVAYWYILSIGAQTDFL

SEQ ID NO: 33 - protein, 15 aa, Homo sapiens
  Immunogenic cluster identified in FVIII
ETVFMSMENPGLWIL

SEQ ID NO: 34 - protein, 16 aa, Homo sapiens
  Immunogenic cluster identified in FVIII
ISAYLLSKNNAIEPRS

SEQ ID NO: 35 - protein, 15 aa, Homo sapiens
  Immunogenic cluster identified in FVIII
PRSFQKKTRHYFIAA

SEQ ID NO: 36 - protein, 16 aa, Homo sapiens
  Immunogenic cluster identified in FVIII
MVTFRNQASRPYSFYS

SEQ ID NO: 37 - protein, 16 aa, Homo sapiens
  Immunogenic cluster identified in FVIII
KTYFWKVQHHMAPTKD

SEQ ID NO: 38 - protein, 21 aa, Homo sapiens
  Immunogenic cluster identified in FVIII
DPTFKENYRFHAINGYIMDTL

SEQ ID NO: 39 - protein, 19 aa, Homo sapiens
  Immunogenic cluster identified in FVIII
DQRIRWYLLSMGSNENIHS

SEQ ID NO: 40 - protein, 16 aa, Homo sapiens
  Immunogenic cluster identified in FVIII
MSTLFLVYSNKCQTPL

SEQ ID NO: 41 - protein, 19 aa, Homo sapiens
  Immunogenic cluster identified in FVIII
PKLARLHYSGSINAWSTKE

SEQ ID NO: 42 - protein, 19 aa, Homo sapiens
  Immunogenic cluster identified in FVIII
SSLYISQFIIMYSLDGKKW

SEQ ID NO: 43 - protein, 18 aa, Homo sapiens
  Immunogenic cluster identified in FVIII
GKKWQTYRGNSTGTLMVF

SEQ ID NO: 44 - protein, 17 aa, Homo sapiens
  Immunogenic cluster identified in FVIII
IARYIRLHPTHYSIRST

SEQ ID NO: 45 - protein, 15 aa, Homo sapiens
  Immunogenic cluster identified in FVIII
SSYFTNMFATWSPSK

SEQ ID NO: 46 - protein, 17 aa, Homo sapiens
  Immunogenic cluster identified in FVIII
KARLHLQGRSNAWRPQV

SEQ ID NO: 47 - protein, 17 aa, Homo sapiens
  Immunogenic cluster identified in FVIII
WLQVDFQKTMKVTGVTT

SEQ ID NO: 48 - protein, 19 aa, Homo sapiens
  Immunogenic cluster identified in FVIII
TSMYVKEFLISSSQDGHQW

SEQ ID NO: 49 - protein, 19 aa, Homo sapiens
  Immunogenic cluster identified in FVIII
QDSFTPVVNSLDPPLLTRY

SEQ ID NO: 50 - protein, 15 aa, Homo sapiens
  Immunogenic cluster identified in FVIII
PQSWVHQIALRMEVL

SEQ ID NO: 51 - protein, 1533 aa, Artificial Sequence
  SIGNAL 1..19
  FVIII-A1A2-3M
MQIELSTCFFLCLLRFCFSATRRYYLGAVELSWDYMQSDLGELPVDARFPPRVPKSFPFNTSVVYKKTLFVEFTDHLFNIAKPRPPWMGLLGPTIQAEVYDTVVITLKNMASHPVSLHAVGVSYWKASEGAEYDDQTSQREKEDDKVFPGGSHTYVWQVLKENGPMASDPLCLTYSYLSHVDLVKDLNSGLIGALLVCREGSLAKEKTQTLHKFILLFAVFDEGKSWHSETKNSLMQDRDAASARAWPKMHTVNGYVNRSLPGLIGCHRKSVYWHVIGMGTTPEVHSIFLEGHTFLVRDHRQASLEISPITFLTAQTLLMDLGQFLLFCHISSHQHDGMEAYVKVDSCPEEPQLRMKNNEEAEDYDDDLTDSEMDVVRFDDDNSPSFIQIRSVAKKHPKTWVHYIAAEEEDWDYAPLVLAPDDRSHKSQYLNNGPQRIGRKYKKVRFMAYTDETFKTREAIQHESGILGPLLYGEVGDTLLIIFKNQASRPYNIYPHGITDVRPLYERRLPKGVKHLKDFPILPGEIFKYKWTVTVEDGPTKSDPRCLTRYYSSFVNMERDLASGLIGPLLICYKESVDQRGNQIMSDKRNVILFSVFDENRSWYLTENIQRFLPNPAGVQLEDPEFQASNIMHSINGYVFDSLQLSVCLHEVAYWYILSIGAQTDFLSVFFSGYTFKHKMVYEDTLTLFPFSGETVFMSMENPGLWILGCHNSDFRNRGMTALLKVSSCDKNTGDYYEDSYEDISAYLLSKNNAIEPRSFSQDPLAWDNHYGTQIPKEEWKSQEKSPEKTAFKKKDTILSLNACESNHAIAAINEGQNKPEIEVTWAKQGRTERLCSQNPPVLKRHQREITRTTLQSDQEEIDYDDTISVEMKKEDFDIYDEDENQSPRSFQKKTRHYFIAAVERLWDYGMSSSPHVLRNRAQSGSVPQFKKVVFQEFTDGSFTQPLYRGELNEHLGLLGPYIRAEVEDNIMVTFRNQASRPYSFYSSLISYEEDQRQGAEPRKNFVKPNETKTYFWKVQHHMAPTKDEFDCKAWAYFSDVDLEKDVHSGLIGPLLVCHTNTLNPAHGRQVTVQEFALFFTIFDETKSWYFTENMERNCRAPCNIQMEDPTFKENYRFHAINGYIMDTLPGLVMAQDQRIRWYLLSMGSNENIHSIHFSGHVFTVRKKEEYKMALYNLYPGVFETVEMLPSKAGIWRVECLIGEHLHAGMSTLFLVYSNKCQTPLGMASGHIRDFQITASGQYGQWAPKLARLHYSGSINAWSTKEPFSWIKVDLLAPMIIHGIKTQGARQKFSSLYISQFIIMYSLDGKKWQTYRGNSTGTLMVFFGNVDSSGIKHNIFNPPIIARYIRLHPTHYSIRSTLRMELMGCDLNSCSMPLGMESKAISDAQITASSYFTNMFATWSPSKARLHLQGRSNAWRPQVNNPKEWLQVDFQKTMKVTGVTTQGVKSLLTSMYVKEFLISSSQDGHQWTLFFQNGKVKVFQGNQDSFTPVVNSLDPPLLTRYLRIHPQSWVHQIALRMEVLGCEAQDLY

SEQ ID NO: 52 - DNA, 4605 bp, Artificial Sequence
  FVIII-19M na
atgcagatcgagctgtctacctgcttcttcctgtgcctgctgcggttctgcttcagcgccacccggcggtactacctgggcgccgtggaactgagctgggactacatgcagagcgacctgggcgagctgcccgtggacgccagattccccccaagagtgcccaagagcttccccttcaacacctccgtggtgtacaagaaaaccctgttcgtcgagttcaccgaccacctgttctccatcgccaagcccagacccccctggatgggcctgctgggccctacaatccaggccgaggtgtacgacaccgtggtcatcaccctgaagaacatggccacccaccccgtgtccctgcacgccgtgggcgtgtcctactggaaggccagcgagggcgccgagtacgacgaccagaccagccagcgcgagaaagaggacgacaaagtctttcctggcggcagccatacctacgtgtggcaggtctccaaagaaaacggccccatggcctccgacccccagtgcctgacctacagctacctgagccacgtggacctggccaaggacctgaacagcggcctgatcggcgccctgctcgtgtgcagagagggcagcctggccaaagagaaaacccagaccctgcacaagttcatcctgctgttcgccgtgttcgacgagggcaagagctggcacagcgagacaaaggacagcctgatgcaggaccgggacgccgcctctgccagagcctggcctaagatgcacaccgtgaacggctacgtgaacagaagcctgcccggactgaccggctgccaccggaagtccgtgtactggcacgtgatcggcatgggtaccacccccgaggtgcacagcatctttctggaaggacacaccttcctcgtgcgggaccaccggcaggccagcctggaaatcagccctatcaccttcctgaccgcccagacactgctgatggacctgggccagttcctgctgttttgccacatcagcagccaccagcacgacggcatggaagcctacgtgaaggtggacagctgccccgaggaaccccagctgcggatgaagaacaacgaggaagccgaggactacgacgacgacctgaccgacagcgagatggacgtcgtcagattcgatgacgacaacagccccagcttcatccagatcagaagcgtggccaagaagcaccccaagacctgggtgcactatatcgccgccgaggaagaggactgggactacgcccctctggtgctggcccccgacgacagaagccacaagagccagtacctgaacaatggcccccagcggatcggccggaagtacaagaaagtgcggttcatggcctacaccgacgagacattcaagaccagagaggccatccagcacgagagcggcatcctgggccccctgctgtacggcgaagtgggcgacaccctgctgattatcttcaagaaccaggccagccggccctacaacatctacccccacggcatcaccgacgtgcggcccctgtacgagagacggctgcccaagggcgtgaagcacctgaaggacttccccatcctgcccggggagatcttcaagtacaagtggaccgtgaccgtggaagatggccccaccaagagcgaccccagatgcctgacccggtactacagcagccacgtgaacatggaacgggacctggcctccgggctgatcggccctctgctgatctgctacaaagaaagcgtggaccagcggggcaaccagatcatgagcgacaagcggaacgtgatcctgttcagcgtgttcgatgagaacagaagctggtatctgaccgagaatatccagcggttcctgcccgagcctgccggcgtgcagctggaagatcccgagttccaggccagcaacatcatgcactccatcaatggctacgtgttcgacagcctgcagctgagcgtgtgcctgcacgaggtggcctactggtacatcctgagcatcggcgcccagaccgacttcctgagcgtgttcttcagcggctacaccttcaagcacaagatggtgtacgaggataccctgaccctgttccccttctccggcgaaaccgtgttcatgagcatggaaaaccccggcaactggattctgggctgccacaacagcgacttccggaaccggggcatgaccgccctgctgaaggtgtccagctgcgacaagaacaccggcgactactacgaggacagctacgaggatatcagcgccagcctgctgagcaagaacaacgccatcgagcctcggagcttctcccaggatcctctggcctgggacaaccactacggcacccagatccccaaagaggaatggaagtcccaggaaaagagccccgagaaaaccgccttcaagaagaaggacaccatcctgagcctgaacgcctgcgagagcaaccacgccattgccgccatcaacgagggccagaacaagcccgagatcgaagtgacctgggctaagcagggccggaccgagagactgtgcagccagaacccccccgtgctgaagcggcaccagagagagatcacccggaccaccctgcagagcgaccaggaagagatcgactacgacgacaccatcagcgtcgagatgaagaaagaggacttcgacatctacgacgaggacgagaaccagagcccccggtccttccagaagaaaacccggcactactttatcgccgccgtggaacggctgtgggactacggcatgagcagcagcccccacgtgctgcggaatagagcccagagcggcagcgtgccccagttcaagaaagtggtgttccaggagttcaccgacggcagcttcacccagcctctgtaccggggcgagctgaacgagcacctgggcctgctgggcccctacatccgggccgaggtggaagataacatcatggtcaccttccggaaccaggccagccggccctacagcttctacagcagcctgatctcctacgaagaggaccagcggcagggcgccgagccccggaagaacttcgtgaagcccaacgagacaaagacctacttctgggaggtgcagcaccacatggcccccaccaaggacgaattcgactgcaaggcctgggcctacttcagcgacgtggacctggaaaaggacgtgcacagcggcctgatcggccccctgctcgtgtgccacaccaacaccctgaaccccgcccacggccggcaggtcacagtgcaggaatttgccctgttcttcaccatcttcgacgagactaagagctggtacttcaccgagaacatggaacggaactgcagagccccctgcaacatccagatggaagatcccaccttcaaagagaactaccggttccacgccatcaatggctacatcatggacaccctgcccggcctggtcatggcccaggaccagagaatccggtggtatctgctgagcatgggcagcaacgagaacatccacagcatccacttcagcggccacgtgttcaccgtgcggaagaaagaagagtacaagatggccctgtacaacctgtaccccggcgtgttcgagacagtggaaatgctgcccagcaaggccggcatctggcgggtggaatgtctgatcggcgagcatctgcacgccggcatgtccaccctgtttctggtgtacagcgacaagtgccagacccccctgggcatggccagcggccacatccgggatttccagatcaccgcctccggccagtacggccagtgggcccctaaactggcccggctgcactacagcggcggcatcaacgcctggtccaccaaagagcccttcagctggatcaaggtggacctgctggcccccatgattatccacggcatcaagacacagggcgccagacagaagttcagcagcctgtacatcagccagttcatcatcatgtacagcctggatggcaagaagtggcagacctaccggggcaacagcaccggcaccctgatggtgttcttcggcaacgtggacagcagcggcatcaagcacaacatcttcaacccccccatcattgcccggtacatccggctgcaccccacccactacagcatccggtccaccctgcggatggaactgatgggctgcgacctgaacagctgctccatgcctctgggcatggaaagcaaggccatcagcgacgcccagatcacagccagcagctacttcaccaacatgttcgccacctggtccccatccaaggccagactgcatctgcagggcagaagcaatgcctggcggcctcaggtcaacaaccccaaagaatggctccaggtggacttccagaaaaccatgaaggtcacaggcgtgaccacccagggcgtgaagtccctgctgacctctatgtacgtgaaagagttcctgatctccagcagccaggacggccaccagtggaccctgttctttcagaacggcaaagtgaaagtgttccagggcaaccaggactccttcacccccgtggtcaacaccctggaccccccactgctgaccagatacctgagaatccacccccagagctgggcccaccagatcgccctgagaatggaagtgctgggatgcgaggcccaggatctgtactgatag

SEQ ID NO: 53 - DNA, 4605 bp, Artificial Sequence
  FVIII-6rs na
atgcagatcgagctgtctacctgcttcttcctgtgcctgctgcggttctgcttcagcgccacccggcggtactacctgggcgccgtggaactgagctgggactacatgcagagcgacctgggcgagctgcccgtggacgccagattccccccaagagtgcccaagagcttccccttcaacacctccgtggtgtacaagaaaaccctgttcgtcgagttcaccgaccacctgttcaatatcgccaagcccagacccccctggatgggcctgctgggccctacaatccaggccgaggtgtacgacaccgtggtcatcaccctgaagaacatggccagccaccccgtgtccctgcacgccgtgggcgtgtcctactggaaggccagcgagggcgccgagtacgacgaccagaccagccagcgcgagaaagaggacgacaaagtctttcctggcggcagccatacctacgtgtggcaggtcctgaaagaaaacggccccatggcctccgaccccctgtgcctgacctacagctacctgagccacgtggacctggtcaaggacctgaacagcggcctgatcggcgccctgctcgtgtgcagagagggcagcctggccaaagagaaaacccagaccctgcacaagttcatcctgctgttcgccgtgttcgacgagggcaagagctggcacagcgagacaaagaacagcctgatgcaggaccgggacgccgcctctgccagagcctggcctaagatgcacaccgtgaacggctacgtgaacagaagcctgcccggactgatcggctgccaccggaagtccgtgtactggcacgtgatcggcatgggtaccacccccgaggtgcacagcatctttctggaaggacacaccttcctcgtgcggaaccaccggcaggccagcctggaaatcagccctatcaccttcctgaccgcccagacactgctgatggacctgggccagttcctgctgttttgccacatcagcagccaccagcacgacggcatggaagcctacgtgaaggtggacagctgccccgaggaaccccagctgcggatgaagaacaacgaggaagccgaggactacgacgacgacctgaccgacagcgagatggacgtcgtcagattcgatgacgacaacagccccagcttcatccagatcagaagcgtggccaagaagcaccccaagacctgggtgcactatatcgccgccgaggaagaggactgggactacgcccctctggtgctggcccccgacgacagaagctacaagagccagtacctgaacaatggcccccagcggatcggccggaagtacaagaaagtgcggttcatggcctacaccgacgagacattcaagaccagagaggccatccagcacgagagcggcatcctgggccccctgctgtacggcgaagtgggcgacaccctgctgattatcttcaagaaccaggccagccggccctacaacatctacccccacggcatcaccgacgtgcggcccctgtacagcagacggctgcccaagggcgtgaagcacctgaaggacttccccatcctgcccggggagatcttcaagtacaagtggaccgtgaccgtggaagatggccccaccaagagcgaccccagatgcctgacccggtactacagcagcttcgtgaacatggaacgggacctggcctccgggctgatcggccctctgctgatctgctacaaagaaagcgtggaccagcggggcaaccagatcatgagcgacaagcggaacgtgatcctgttcagcgtgttcgatgagaacagaagctggtatctgaccgagaatatccagcggttcctgcccaaccctgccggcgtgcagctggaagatcccgagttccaggccagcaacatcatgcactccatcaatggctacgtgttcgacagcctgcagctgagcgtgtgcctgcacgaggtggcctactggtacatcctgagcatcggcgcccagaccgacttcctgagcgtgttcttcagcggctacaccttcaagcacaagatggtgtacgaggataccctgaccctgttccccttctccggcgaaaccgtgttcatgagcatggaaaaccccggcctgtggattctgggctgccacaacagcgacttccggaaccggggcatgaccgccctgctgaaggtgtccagctgcgacaagaacaccggcgactactacgaggacagctacgaggatatcagcgcctacctgctgagcaagaacaacgccatcgagcctcggagcttctcccaggatcctctggcctgggacaaccactacggcacccagatccccaaagaggaatggaagtcccaggaaaagagccccgagaaaaccgccttcaagaagaaggacaccatcctgagcctgaacgcctgcgagagcaaccacgccattgccgccatcaacgagggccagaacaagcccgagatcgaagtgacctgggctaagcagggccggaccgagagactgtgcagccagaacccccccgtgctgaagcggcaccagagagagatcacccggaccaccctgcagagcgaccaggaagagatcgactacgacgacaccatcagcgtcgagatgaagaaagaggacttcgacatctacgacgaggacgagaaccagagcccccggtccttccagaagaaaacccggcactactttatcgccgccgtggaacggctgtgggactacggcatgagcagcagcccccacgtgctgcggaatagagcccagagcggcagcgtgccccagttcaagaaagtggtgttccaggagttcaccgacggcagcttcacccagcctctgtaccggggcgagctgaacgagcacctgggcctgctgggcccctacatccgggccgaggtggaagataacatcatggtcaccttccggaaccaggccagccggccctacagcttctacagcagcctgatctcctacgaagaggaccagcggcagggcgccgagccccggaagaacttcgtgaagcccaacgagacaaagacctacttctggaaggtgcagcaccacatggcccccaccaaggacgaattcgactgcaaggcctgggcctacttcagcgacgtggacctggaaaaggacgtgcacagcggcctgatcggccccctgctcgtgtgccacaccaacaccctgaaccccgcccacggccggcaggtcacagtgcaggaatttgccctgttcttcaccatcttcgacgagactaagagctggtacttcaccgagaacatggaacggaactgcagagccccctgcaacatccagatggaagatcccaccttcaaagagaactaccggttccacgccatcaatggctacatcatggacaccctgcccggcctggtcatggcccaggaccagagaatccggtggtatctgctgagcatgggcagcaacgagaacatccacagcatccacttcagcggccacgtgttcaccgtgcggaagaaagaagagtacaagatggccctgtacaacctgtaccccggcgtgttcgagacagtggaaatgctgcccagcaaggccggcatctggcgggtggaatgtctgatcggcgagcatctgcacgccggcatgtccaccctgtttctggtgtacagcaacaagtgccagacccccctgggcatggccagcggccacatccgggatttccagatcaccgcctccggccagtacggccagtgggcccctaaactggcccggctgcactacagcggcagcatcaacgcctggtccaccaaagagcccttcagctggatcaaggtggacctgctggcccccatgattatccacggcatcaagacacagggcgccagacagaagttcagcagcctgtacatcagccagttcatcatcatgtacagcctggatggcaagaagtggcagacctaccggggcaacagcaccggcaccctgatggtgttcttcggcaacgtggacagcagcggcatcaagcacaacatcttcaacccccccatcattgcccggtacatccggctgcaccccacccactacagcatccggtccaccctgcggatggaactgatgggctgcgacctgaacagctgctccatgcctctgggcatggaaagcaaggccatcagcgacgcccagatcacagccagcagctacttcaccaacatgttcgccacctggtccccatccaaggccagactgcatctgcagggcagaagcaatgcctggcggcctcaggtcaacaaccccaaagaatggctccaggtggacttccagaaaaccatgaaggtcacaggcgtgaccacccagggcgtgaagtccctgctgacctctatgtacgtgaaagagttcctgatctccagcagccaggacggccaccagtggaccctgttctttcagaacggcaaagtgaaagtgttccagggcaaccaggactccttcacccccgtggtcaactccctggaccccccactgctgaccagatacctgagaatccacccccagagctgggtgcaccagatcgccctgagaatggaagtgctgggatgcgaggcccaggatctgtactgatag

SEQ ID NO: 54 - protein, 16 aa, Artificial Sequence
  Immunogenic cluster identified in FVIII
GEHLHAGMSTLFLVYS